European Patent Specification EP 3 069 606 B1, published January 4, 2023. Title: Interleukin 2 receptor gamma gene targeting vector, production of SCID-like miniature pigs by TALEN-mediated gene targeting and use thereof. Applicant: Konkuk University Industrial Cooperation Corp. The sequence listing filed with the application follows.

SEQUENCE LISTING (21 sequences)

SEQ ID NO: 1 - DNA, 50 bp, Sus scrofa
tcagtgttttgtgttcaatgttgagtacatgaattgcacttggaacagca

SEQ ID NO: 2 - DNA, 24 bp, Artificial Sequence
  primer
ctggactattagaaggatgtgggc

SEQ ID NO: 3 - DNA, 24 bp, Artificial Sequence
  primer
atatagtgggaagcctgggatgct

SEQ ID NO: 4 - DNA, 22 bp, Artificial Sequence
  primer
cgtttgttaaaactgcagcata

SEQ ID NO: 5 - DNA, 20 bp, Artificial Sequence
  primer
ttttgcttccctttccttcc

SEQ ID NO: 6 - DNA, 20 bp, Artificial Sequence
  primer
agccagaggaaggggtttta

SEQ ID NO: 7 - DNA, 20 bp, Artificial Sequence
  primer
ggttaaccagctcaggcaac

SEQ ID NO: 8 - DNA, 20 bp, Artificial Sequence
  primer
gtctggttgcagctcaaggt

SEQ ID NO: 9 - DNA, 22 bp, Artificial Sequence
  primer
gccactgtggactctagaggat

SEQ ID NO: 10 - DNA, 20 bp, Artificial Sequence
  primer
attcacacaggggagaaacg

SEQ ID NO: 11 - DNA, 20 bp, Artificial Sequence
  primer
gtggaaatttttcccccatt

SEQ ID NO: 12 - DNA, 19 bp, Artificial Sequence
  primer
ctttggacctgcccacttt

SEQ ID NO: 13 - DNA, 20 bp, Artificial Sequence
  primer
ggatgtgtgatcggttccat

SEQ ID NO: 14 - DNA, 20 bp, Artificial Sequence
  primer
tgagggagagaggagacctg

SEQ ID NO: 15 - DNA, 20 bp, Artificial Sequence
  primer
ctaggggaaggaaagggatg

SEQ ID NO: 16 - DNA, 20 bp, Artificial Sequence
  primer
ggcgtacatgcctaccatct

SEQ ID NO: 17 - DNA, 19 bp, Artificial Sequence
  primer
ctgtccacggtctttgtgg

SEQ ID NO: 18 - DNA, 20 bp, Artificial Sequence
  primer
ttctcccaaccccatttaca

SEQ ID NO: 19 - DNA, 20 bp, Artificial Sequence
  primer
cctgagttgaaccagcacct

SEQ ID NO: 20 - DNA, 25 bp, Artificial Sequence
  primer
aaaaagttcttcctgttttgacaga

SEQ ID NO: 21 - DNA, 20 bp, Artificial Sequence
  primer
tggttattccaccaatgcaa